European Patent Specification EP 3 247 396 B1, published August 28, 2024. Title: Methods and Compositions for the Treatment of Diseases and Disorders. Applicant: Thomas, Sunil Mullin, James Prendergast, George C. The sequence listing filed with the application follows.

SEQUENCE LISTING (2 sequences)

SEQ ID NO: 1 - protein, 451 aa, Homo sapiens
MLWNVVTAGKIASNVQKKLTRAQEKVLQKLGKADETKDEQFEQCVQNFNKQLTEGTRLQKDLRTYLASVKAMHEASKKLNECLQEVYEPDWPGRDEANKIAENNDLLWMDYHQKLVDQALLTMDTYLGQFPDIKSRIAKRGRKLVDYDSARHHYESLQTAKKKDEAKIAKAEEELIKAQKVFEEMNVDLQEELPSLWNSRVGFYVNTFQSIAGLEENFHKEMSKLNQNLNDVLVGLEKQHGSNTFTVKAQPRKKSKLFSRLRRKKNSDNAPAKGNKSPSPPDGSPAATPEIRVNHEPEPAGGATPGATLPKSPSQPAEASEVAGGTQPAAGAQEPGETAASEAASSSLPAVVVETFPATVNGTVEGGSGAGRLDLPPGFMFKVQAQHDYTATDTDELQLKAGDVVLVIPFQNPEEQDEGWLMGVKESDWNQHKKLEKCRGVFPENFTERVP

SEQ ID NO: 2 - protein, 34 aa, Artificial Sequence
  Bin1 fragment
AGGTQPAAGAQEPGETAASEAASSSLPAVVVETF